European Patent Specification EP 3 472 194 B1, published July 1, 2026. Title: Optimized Mini-dystrophin Genes and Expression Cassettes and Their Use. Applicant: Bamboo Therapeutics, Inc. The University of North Carolina at Chapel Hill. The sequence listing filed with the application follows.

SEQUENCE LISTING (28 sequences)

SEQ ID NO: 1 - DNA, 3978 bp, Artificial Sequence
  Hopti-Dys3978 gene
atgctttggtgggaggaagtggaggactgctacgagagagaggacgtgcagaagaaaaccttcaccaagtgggtgaacgcccagttcagcaagttcggcaagcagcacatcgagaacctgttcagcgacctgcaggatggcaggagactgctggacctgctggagggcctgaccggccagaagctgcccaaggagaagggcagcaccagagtgcacgccctgaacaacgtgaacaaggccctgagagtgctgcagaacaacaacgtggacctggtgaacatcggcagcaccgacatcgtggacggcaaccacaagctgaccctgggcctgatctggaacatcatcctgcactggcaggtgaagaacgtgatgaagaacatcatggccggcctgcagcagaccaacagcgagaagatcctgctgagctgggtgaggcagagcaccagaaactacccccaggtgaacgtgatcaacttcaccacctcctggagcgacggcctggccctgaacgccctgatccacagccacagacccgacctgttcgactggaacagcgtggtgtgtcagcagagcgccacccagagactggagcacgccttcaacatcgccagataccagctgggcatcgagaagctgctggaccccgaggacgtggacaccacctaccccgacaagaaaagcatcctcatgtacattaccagcctgttccaggtgctgccccagcaggtgtccatcgaggccatccaggaagtggaaatgctgcccaggccccccaaagtgaccaaggaggagcacttccagctgcaccaccagatgcactacagccagcagatcacagtgagcctggcccagggctatgagagaaccagcagccccaagcccagattcaagagctacgcctacacccaggccgcctacgtgaccacctccgaccccaccagaagccccttccccagccagcacctggaggcccccgaggacaagagcttcggcagcagcctgatggagagcgaagtgaacctggacagataccagaccgccctggaggaagtgctgtcctggctgctgagcgccgaggacaccctgcaggcccagggcgagatcagcaacgacgtggaagtggtgaaggaccagttccacacccacgagggctacatgatggatctgaccgcccaccagggcagagtgggcaatatcctgcagctgggcagcaagctgatcggcaccggcaagctgagcgaggacgaggagaccgaagtgcaggagcagatgaacctgctgaacagcagatgggagtgcctgagagtggccagcatggagaagcagagcaacctgcacagagtgctgatggacctgcagaaccagaagctgaaggagctgaacgactggctgaccaagaccgaggagcggaccagaaagatggaggaggagcccctgggccccgacctggaggacctgaagagacaggtgcagcagcacaaagtgctgcaggaggacctggagcaggagcaggtgcgcgtgaacagcctgacccacatggtggtggtcgtggacgagagcagcggcgaccacgccacagccgccctggaagagcagctgaaagtgctgggcgacagatgggccaatatttgtaggtggaccgaggacagatgggtgctgctgcaggaccagcccgacctggcccctggcctgaccaccatcggcgccagccccacccagaccgtgaccctggtgacccagcccgtggtgacaaaggagaccgccatcagcaagctggagatgcccagctccctgatgctggaagtgcccacccaccgcctgctccagcagttccccctggacctggagaagttcctggcctggctgaccgaggccgaaaccaccgccaatgtgctccaggacgccactagaaaggagaggctgctggaggacagcaagggcgtgaaagagctgatgaagcagtggcaggatctgcagggcgaaatcgaggcccacaccgacgtgtaccacaacctggacgagaacagccagaagattctgaggagcctggagggcagcgacgacgccgtcctgctccagaggaggctggacaacatgaacttcaagtggagcgagctgcggaagaagagcctgaacatccggagccacctggaagccagcagcgaccagtggaagagactgcacctgagcctgcaggagctgctggtgtggctgcagctgaaggacgacgagctgagcagacaggcccccatcggcggcgacttccccgccgtgcagaagcagaacgacgtgcaccgggccttcaagagggagctgaaaaccaaggaacccgtgatcatgagcaccctggagacagtgcggatcttcctgaccgagcagcccctggagggactggagaagctgtaccaggagcccagagagctgccccccgaggagagagcccagaacgtgaccaggctgctgagaaagcaggccgaggaagtgaataccgagtgggagaagctgaatctgcacagcgccgactggcagagaaagatcgacgagaccctggagagactccaggaactgcaggaagccaccgacgagctggacctgaagctgagacaggccgaagtgatcaagggcagctggcagcctgtgggcgatctgctgatcgactccctgcaggatcacctggagaaagtgaaggccctgcggggcgagatcgcccccctgaaggagaatgtgagccacgtgaacgacctggccagacagctgaccaccctgggcatccagctgagcccctacaacctgagcacactggaggatctgaacacccggtggaaactgctgcaggtggccgtggaggatagagtgaggcagctgcacgaagcccacagagacttcggccctgcctcccagcacttcctgagcaccagcgtgcagggcccctgggagagagccatctcccccaacaaagtgccctactacatcaaccacgagacccagaccacctgctgggaccaccctaagatgaccgagctgtatcagagcctggccgacctgaacaatgtgcggttcagcgcctacagaaccgccatgaagctgcggagactgcagaaggccctgtgcctggatctgctgagcctgagcgccgcctgcgacgccctggaccagcacaacctgaagcagaatgaccagcccatggacatcctgcagatcatcaactgcctgaccacaatctacgaccggctggaacaggagcacaacaacctggtgaatgtgcccctgtgcgtggacatgtgcctgaattggctgctgaacgtgtacgacaccggcaggaccggcagaatccgcgtgctgagcttcaagaccggcatcatcagcctgtgcaaggcccacctggaggataagtaccgctacctgttcaagcaggtggccagcagcaccggcttctgcgatcagaggagactgggcctgctgctgcacgatagcatccagatccctaggcagctgggcgaagtggccagctttggcggcagcaacatcgagccctctgtgaggagctgcttccagttcgccaacaacaagcccgagatcgaggccgccctgttcctggactggatgaggctggagcctcagagcatggtgtggctgcctgtgctgcacagagtggccgccgccgagaccgccaagcaccaggccaagtgcaatatctgcaaggagtgccccatcatcggcttccggtacaggagcctgaagcacttcaactacgacatctgccagagctgctttttcagcggcagagtggccaagggccacaaaatgcactaccccatggtggagtactgcacccccaccacctccggcgaggatgtgagagacttcgccaaagtgctgaagaataagttccggaccaagcggtactttgccaagcaccccaggatgggctacctgcccgtgcagaccgtgctggaaggcgacaacatggagacctga

SEQ ID NO: 2 - DNA, 3837 bp, Artificial Sequence
  Hopti-Dys3837 gene
atgctttggtgggaggaagtggaggactgctacgagagagaggacgtgcagaagaaaaccttcaccaagtgggtgaacgcccagttcagcaagttcggcaagcagcacatcgagaacctgttcagcgacctgcaggatggcaggagactgctggacctgctggagggcctgaccggccagaagctgcccaaggagaagggcagcaccagagtgcacgccctgaacaacgtgaacaaggccctgagagtgctgcagaacaacaacgtggacctggtgaacatcggcagcaccgacatcgtggacggcaaccacaagctgaccctgggcctgatctggaacatcatcctgcactggcaggtgaagaacgtgatgaagaacatcatggccggcctgcagcagaccaacagcgagaagatcctgctgagctgggtgaggcagagcaccagaaactacccccaggtgaacgtgatcaacttcaccacctcctggagcgacggcctggccctgaacgccctgatccacagccacagacccgacctgttcgactggaacagcgtggtgtgtcagcagagcgccacccagagactggagcacgccttcaacatcgccagataccagctgggcatcgagaagctgctggaccccgaggacgtggacaccacctaccccgacaagaaaagcatcctcatgtacattaccagcctgttccaggtgctgccccagcaggtgtccatcgaggccatccaggaagtggaaatgctgcccaggccccccaaagtgaccaaggaggagcacttccagctgcaccaccagatgcactacagccagcagatcacagtgagcctggcccagggctatgagagaaccagcagccccaagcccagattcaagagctacgcctacacccaggccgcctacgtgaccacctccgaccccaccagaagccccttccccagccagcacctggaggcccccgaggacaagagcttcggcagcagcctgatggagagcgaagtgaacctggacagataccagaccgccctggaggaagtgctgtcctggctgctgagcgccgaggacaccctgcaggcccagggcgagatcagcaacgacgtggaagtggtgaaggaccagttccacacccacgagggctacatgatggatctgaccgcccaccagggcagagtgggcaatatcctgcagctgggcagcaagctgatcggcaccggcaagctgagcgaggacgaggagaccgaagtgcaggagcagatgaacctgctgaacagcagatgggagtgcctgagagtggccagcatggagaagcagagcaacctgcacagagtgctgatggacctgcagaaccagaagctgaaggagctgaacgactggctgaccaagaccgaggagcggaccagaaagatggaggaggagcccctgggccccgacctggaggacctgaagagacaggtgcagcagcacaaagtgctgcaggaggacctggagcaggagcaggtgcgcgtgaacagcctgacccacatggtggtggtcgtggacgagagcagcggcgaccacgccacagccgccctggaagagcagctgaaagtgctgggcgacagatgggccaatatttgtaggtggaccgaggacagatgggtgctgctgcaggacacccaccgcctgctccagcagttccccctggacctggagaagttcctggcctggctgaccgaggccgaaaccaccgccaatgtgctccaggacgccactagaaaggagaggctgctggaggacagcaagggcgtgaaagagctgatgaagcagtggcaggatctgcagggcgaaatcgaggcccacaccgacgtgtaccacaacctggacgagaacagccagaagattctgaggagcctggagggcagcgacgacgccgtcctgctccagaggaggctggacaacatgaacttcaagtggagcgagctgcggaagaagagcctgaacatccggagccacctggaagccagcagcgaccagtggaagagactgcacctgagcctgcaggagctgctggtgtggctgcagctgaaggacgacgagctgagcagacaggcccccatcggcggcgacttccccgccgtgcagaagcagaacgacgtgcaccgggccttcaagagggagctgaaaaccaaggaacccgtgatcatgagcaccctggagacagtgcggatcttcctgaccgagcagcccctggagggactggagaagctgtaccaggagcccagagagctgccccccgaggagagagcccagaacgtgaccaggctgctgagaaagcaggccgaggaagtgaataccgagtgggagaagctgaatctgcacagcgccgactggcagagaaagatcgacgagaccctggagagactccaggaactgcaggaagccaccgacgagctggacctgaagctgagacaggccgaagtgatcaagggcagctggcagcctgtgggcgatctgctgatcgactccctgcaggatcacctggagaaagtgaaggccctgcggggcgagatcgcccccctgaaggagaatgtgagccacgtgaacgacctggccagacagctgaccaccctgggcatccagctgagcccctacaacctgagcacactggaggatctgaacacccggtggaaactgctgcaggtggccgtggaggatagagtgaggcagctgcacgaagcccacagagacttcggccctgcctcccagcacttcctgagcaccagcgtgcagggcccctgggagagagccatctcccccaacaaagtgccctactacatcaaccacgagacccagaccacctgctgggaccaccctaagatgaccgagctgtatcagagcctggccgacctgaacaatgtgcggttcagcgcctacagaaccgccatgaagctgcggagactgcagaaggccctgtgcctggatctgctgagcctgagcgccgcctgcgacgccctggaccagcacaacctgaagcagaatgaccagcccatggacatcctgcagatcatcaactgcctgaccacaatctacgaccggctggaacaggagcacaacaacctggtgaatgtgcccctgtgcgtggacatgtgcctgaattggctgctgaacgtgtacgacaccggcaggaccggcagaatccgcgtgctgagcttcaagaccggcatcatcagcctgtgcaaggcccacctggaggataagtaccgctacctgttcaagcaggtggccagcagcaccggcttctgcgatcagaggagactgggcctgctgctgcacgatagcatccagatccctaggcagctgggcgaagtggccagctttggcggcagcaacatcgagccctctgtgaggagctgcttccagttcgccaacaacaagcccgagatcgaggccgccctgttcctggactggatgaggctggagcctcagagcatggtgtggctgcctgtgctgcacagagtggccgccgccgagaccgccaagcaccaggccaagtgcaatatctgcaaggagtgccccatcatcggcttccggtacaggagcctgaagcacttcaactacgacatctgccagagctgctttttcagcggcagagtggccaagggccacaaaatgcactaccccatggtggagtactgcacccccaccacctccggcgaggatgtgagagacttcgccaaagtgctgaagaataagttccggaccaagcggtactttgccaagcaccccaggatgggctacctgcccgtgcagaccgtgctggaaggcgacaacatggagacctga

SEQ ID NO: 3 - DNA, 3978 bp, Artificial Sequence
  Copti-Dys3978 gene
atgctttggtgggaggaagtggaggactgctacgagcgggaggacgtgcagaagaaaaccttcaccaagtgggtgaacgcccagttcagcaagttcggcaagcagcacatcgagaacctgttcagcgacctgcaggacggcaggcggctgctggacctcctggaaggcctgaccggccagaagctgcccaaagagaagggcagcaccagggtgcacgccctgaacaacgtgaacaaggccctgagggtgctgcagaacaacaacgtggacctggtgaacatcggcagcaccgacatcgtggacggcaaccacaagctgaccctgggcctgatctggaacatcatcctgcactggcaggtcaagaacgtgatgaagaacatcatggccggcctgcagcagaccaacagcgagaagatcctgctgtcctgggtgcggcagagcaccaggaactacccccaggtcaacgtgatcaacttcaccacctcttggagcgacggcctggccctgaacgccctgatccacagccacaggcccgacctgttcgactggaacagcgtggtgtgccagcagagcgccacccagaggctggaacacgccttcaacatcgccagataccagctgggcatcgagaagctgctggatcccgaggacgtggacaccacctaccccgacaagaaaagcatcctcatgtacatcaccagcctgttccaggtgctgccccagcaggtgtccatcgaggccatccaggaagtggagatgctgcccaggccccccaaggtcaccaaagaggaacacttccagctgcaccaccagatgcactacagccagcagatcaccgtgagcctggcccagggctacgagaggaccagcagccccaagcccaggttcaagagctacgcctacacccaggccgcctacgtgaccacctccgaccccaccaggtcccccttccccagccagcatctcgaagcccccgaggacaagagcttcggcagcagcctgatggaaagcgaggtgaacctggacagataccagaccgccctggaagaagtgctgtcttggctgctgtccgccgaggacaccctgcaggcccagggcgagatcagcaacgacgtggaggtcgtgaaggaccagttccacacccacgagggctacatgatggacctgaccgcccaccagggcagagtgggcaacatcctgcagctgggcagcaagctgatcggcaccggcaagctgtccgaggacgaggaaaccgaggtgcaggaacagatgaacctgctgaacagcagatgggagtgcctgagggtggccagcatggaaaagcagagcaacctgcacagggtgctgatggatctgcagaaccagaagctcaaagagctgaacgactggctgaccaagaccgaggaaaggacccggaagatggaagaggaacccctgggccccgatctcgaagatctgaagaggcaggtgcagcagcacaaggtgctgcaggaagatctcgaacaggaacaggtccgggtcaacagcctgacccacatggtcgtggtggtggacgagagcagcggcgaccacgccaccgctgccctggaagagcagctgaaggtgctgggcgacagatgggccaacatctgccggtggaccgaggacagatgggtcctcctgcaggaccagcccgacctggcccctggcctgacaaccatcggcgccagccccacccagaccgtgaccctggtgacccagcccgtggtgaccaaagagaccgccatcagcaagctggaaatgcccagctccctgatgctggaagtgcccacccacaggctcctccagcagttccccctggacctggaaaagttcctggcctggctgaccgaggccgagaccaccgccaacgtgctgcaggacgccaccaggaaagagaggctgctggaagatagcaagggcgtgaaagagctgatgaagcagtggcaggacctgcagggggagattgaggcccacaccgacgtgtaccacaacctggacgagaacagccagaaaatcctgagaagcctggaaggcagcgacgacgccgtgctgctgcagaggcggctggacaacatgaacttcaagtggagcgagctgaggaagaagagcctgaacatcaggtcccatctggaagccagcagcgaccagtggaagaggctgcacctgagcctgcaggaactgctcgtctggctgcagctgaaagacgacgagctgtccaggcaggcccccatcggcggcgacttccccgccgtgcagaaacagaacgacgtgcacagggccttcaagcgggagctgaaaaccaaagagcccgtgatcatgagcaccctggaaaccgtgaggatcttcctgaccgagcagcccctggaaggactggaaaagctgtaccaggaacccagagagctgccccccgaggaacgggcccagaacgtgaccaggctgctgagaaagcaggccgaggaagtgaacaccgagtgggagaagctgaacctgcactccgccgactggcagaggaagatcgacgagaccctggaaaggctccaggaactgcaggaagccaccgacgagctggacctgaagctgagacaggccgaggtgatcaagggcagctggcagcccgtgggcgacctgctgatcgactccctgcaggatcacctggaaaaagtgaaggccctgcggggcgagatcgcccccctgaaagagaacgtcagccacgtcaacgacctggccaggcagctgaccaccctgggcatccagctgtccccctacaacctgtccaccctggaagatctgaacacaaggtggaagctgctgcaggtggccgtggaggacagagtgaggcagctgcacgaggcccacagggacttcggccctgcctcccagcacttcctgagcaccagcgtgcagggcccctgggagagggccatctcccccaacaaggtgccctactacatcaaccacgagacccagaccacctgctgggaccaccctaagatgaccgagctgtaccagtccctggccgacctgaacaatgtgcggttcagcgcctaccggaccgccatgaagctgaggcggctgcagaaagccctgtgcctggatctgctgtccctgagcgccgcctgcgacgccctggaccagcacaacctgaagcagaacgaccagcccatggatatcctgcagatcatcaactgtctgaccaccatctacgacaggctggaacaggaacacaacaacctggtcaacgtgcccctgtgcgtggacatgtgcctgaactggctgctgaacgtgtacgacaccggcaggaccggccggatcagggtgctgtccttcaagaccggcatcatcagcctgtgcaaggcccacctggaagataagtaccgctacctgttcaagcaggtggccagctctaccggcttctgcgaccagcggaggctgggcctgctgctgcacgacagcatccagatcccccggcagctgggcgaggtggcctccttcggcggcagcaacatcgagcccagcgtgcggagctgcttccagttcgccaacaacaagcccgagatcgaggccgccctgttcctggactggatgcggctggaaccccagagcatggtctggctgcccgtgctgcacagagtggctgccgccgagaccgccaagcaccaggccaagtgcaacatctgcaaagagtgccccatcatcggcttcaggtacagaagcctgaagcacttcaactacgacatctgccagagctgtttcttcagcggcagggtggccaagggccacaaaatgcactaccccatggtggagtactgcacccccaccacctccggcgaggacgtgagggacttcgccaaggtgctgaagaataagttccggaccaagcggtacttcgccaaacaccccaggatgggctacctgcccgtgcagaccgtgctggaaggcgacaacatggaaacctga

SEQ ID NO: 4 - DNA, 606 bp, Artificial Sequence
  hCK promoter
gaattcggtaccccactacgggtttaggctgcccatgtaaggaggcaaggcctggggacacccgagatgcctggttataattaacccagacatgtggctgccccccccccccccaacacctgctgcctctaaaaataaccctgtccctggtggatcccctgcatgcgaagatcttcgaacaaggctgtgggggactgagggcaggctgtaacaggcttgggggccagggcttatacgtgcctgggactcccaaagtattactgttccatgttcccggcgaagggccagctgtcccccgccagctagactcagcacttagtttaggaaccagtgagcaagtcagcccttggggcagcccatacaaggccatggggctgggcaagctgcacgcctgggtccggggtgggcacggtgcccgggcaacgagctgaaagctcatctgctctcaggggcccctccctggggacagcccctcctggctagtcacaccctgtaggctcctctatataacccaggggcacaggggctgccctcattctaccaccacctccacagcacagacagacactcaggagccagccagcgtcgagcggccgatccgccacc

SEQ ID NO: 5 - DNA, 759 bp, Artificial Sequence
  hCKplus promoter
gaattcggtaccccactacgggtctaggctgcccatgtaaggaggcaaggcctggggacacccgagatgcctggttataattaaccccaacacctgctgcccccccccccccaacacctgctgcctctaaaaataaccctgtccctggtggatcccctgcatgccccactacgggtttaggctgcccatgtaaggaggcaaggcctggggacacccgagatgcctggttataattaacccagacatgtggctgccccccccccccccaacacctgctgcctctaaaaataaccctgtccctggtggatcccctgcatgcgaagatcttcgaacaaggctgtgggggactgagggcaggctgtaacaggcttgggggccagggcttatacgtgcctgggactcccaaagtattactgttccatgttcccggcgaagggccagctgtcccccgccagctagactcagcacttagtttaggaaccagtgagcaagtcagcccttggggcagcccatacaaggccatggggctgggcaagctgcacgcctgggtccggggtgggcacggtgcccgggcaacgagctgaaagctcatctgctctcaggggcccctccctggggacagcccctcctggctagtcacaccctgtaggctcctctatataacccaggggcacaggggctgccctcattctaccaccacctccacagcacagacagacactcaggagccagccagcgtcgagcggccgatccgccacc

SEQ ID NO: 6 - DNA, 67 bp, Artificial Sequence
  Synthetic polyA
tgaggagctcgagaggcctaataaagagctcagatgcatcgatcagagtgtgttggttttttgtgtg

SEQ ID NO: 7 - protein, 1325 aa, Artificial Sequence
  Dys3978 protein
MLWWEEVEDCYEREDVQKKTFTKWVNAQFSKFGKQHIENLFSDLQDGRRLLDLLEGLTGQKLPKEKGSTRVHALNNVNKALRVLQNNNVDLVNIGSTDIVDGNHKLTLGLIWNIILHWQVKNVMKNIMAGLQQTNSEKILLSWVRQSTRNYPQVNVINFTTSWSDGLALNALIHSHRPDLFDWNSVVCQQSATQRLEHAFNIARYQLGIEKLLDPEDVDTTYPDKKSILMYITSLFQVLPQQVSIEAIQEVEMLPRPPKVTKEEHFQLHHQMHYSQQITVSLAQGYERTSSPKPRFKSYAYTQAAYVTTSDPTRSPFPSQHLEAPEDKSFGSSLMESEVNLDRYQTALEEVLSWLLSAEDTLQAQGEISNDVEVVKDQFHTHEGYMMDLTAHQGRVGNILQLGSKLIGTGKLSEDEETEVQEQMNLLNSRWECLRVASMEKQSNLHRVLMDLQNQKLKELNDWLTKTEERTRKMEEEPLGPDLEDLKRQVQQHKVLQEDLEQEQVRVNSLTHMVVVVDESSGDHATAALEEQLKVLGDRWANICRWTEDRWVLLQDQPDLAPGLTTIGASPTQTVTLVTQPVVTKETAISKLEMPSSLMLEVPTHRLLQQFPLDLEKFLAWLTEAETTANVLQDATRKERLLEDSKGVKELMKQWQDLQGEIEAHTDVYHNLDENSQKILRSLEGSDDAVLLQRRLDNMNFKWSELRKKSLNIRSHLEASSDQWKRLHLSLQELLVWLQLKDDELSRQAPIGGDFPAVQKQNDVHRAFKRELKTKEPVIMSTLETVRIFLTEQPLEGLEKLYQEPRELPPEERAQNVTRLLRKQAEEVNTEWEKLNLHSADWQRKIDETLERLQELQEATDELDLKLRQAEVIKGSWQPVGDLLIDSLQDHLEKVKALRGEIAPLKENVSHVNDLARQLTTLGIQLSPYNLSTLEDLNTRWKLLQVAVEDRVRQLHEAHRDFGPASQHFLSTSVQGPWERAISPNKVPYYINHETQTTCWDHPKMTELYQSLADLNNVRFSAYRTAMKLRRLQKALCLDLLSLSAACDALDQHNLKQNDQPMDILQIINCLTTIYDRLEQEHNNLVNVPLCVDMCLNWLLNVYDTGRTGRIRVLSFKTGIISLCKAHLEDKYRYLFKQVASSTGFCDQRRLGLLLHDSIQIPRQLGEVASFGGSNIEPSVRSCFQFANNKPEIEAALFLDWMRLEPQSMVWLPVLHRVAAAETAKHQAKCNICKECPIIGFRYRSLKHFNYDICQSCFFSGRVAKGHKMHYPMVEYCTPTTSGEDVRDFAKVLKNKFRTKRYFAKHPRMGYLPVQTVLEGDNMET

SEQ ID NO: 8 - protein, 1278 aa, Artificial Sequence
  Dys3837 protein
MLWWEEVEDCYEREDVQKKTFTKWVNAQFSKFGKQHIENLFSDLQDGRRLLDLLEGLTGQKLPKEKGSTRVHALNNVNKALRVLQNNNVDLVNIGSTDIVDGNHKLTLGLIWNIILHWQVKNVMKNIMAGLQQTNSEKILLSWVRQSTRNYPQVNVINFTTSWSDGLALNALIHSHRPDLFDWNSVVCQQSATQRLEHAFNIARYQLGIEKLLDPEDVDTTYPDKKSILMYITSLFQVLPQQVSIEAIQEVEMLPRPPKVTKEEHFQLHHQMHYSQQITVSLAQGYERTSSPKPRFKSYAYTQAAYVTTSDPTRSPFPSQHLEAPEDKSFGSSLMESEVNLDRYQTALEEVLSWLLSAEDTLQAQGEISNDVEVVKDQFHTHEGYMMDLTAHQGRVGNILQLGSKLIGTGKLSEDEETEVQEQMNLLNSRWECLRVASMEKQSNLHRVLMDLQNQKLKELNDWLTKTEERTRKMEEEPLGPDLEDLKRQVQQHKVLQEDLEQEQVRVNSLTHMVVVVDESSGDHATAALEEQLKVLGDRWANICRWTEDRWVLLQDTHRLLQQFPLDLEKFLAWLTEAETTANVLQDATRKERLLEDSKGVKELMKQWQDLQGEIEAHTDVYHNLDENSQKILRSLEGSDDAVLLQRRLDNMNFKWSELRKKSLNIRSHLEASSDQWKRLHLSLQELLVWLQLKDDELSRQAPIGGDFPAVQKQNDVHRAFKRELKTKEPVIMSTLETVRIFLTEQPLEGLEKLYQEPRELPPEERAQNVTRLLRKQAEEVNTEWEKLNLHSADWQRKIDETLERLQELQEATDELDLKLRQAEVIKGSWQPVGDLLIDSLQDHLEKVKALRGEIAPLKENVSHVNDLARQLTTLGIQLSPYNLSTLEDLNTRWKLLQVAVEDRVRQLHEAHRDFGPASQHFLSTSVQGPWERAISPNKVPYYINHETQTTCWDHPKMTELYQSLADLNNVRFSAYRTAMKLRRLQKALCLDLLSLSAACDALDQHNLKQNDQPMDILQIINCLTTIYDRLEQEHNNLVNVPLCVDMCLNWLLNVYDTGRTGRIRVLSFKTGIISLCKAHLEDKYRYLFKQVASSTGFCDQRRLGLLLHDSIQIPRQLGEVASFGGSNIEPSVRSCFQFANNKPEIEAALFLDWMRLEPQSMVWLPVLHRVAAAETAKHQAKCNICKECPIIGFRYRSLKHFNYDICQSCFFSGRVAKGHKMHYPMVEYCTPTTSGEDVRDFAKVLKNKFRTKRYFAKHPRMGYLPVQTVLEGDNMET

SEQ ID NO: 9 - DNA, 4953 bp, Artificial Sequence
  AAV vector genome with Hopti-Dys3978 gene
ttggccactccctctctgcgcgctcgctcgctcactgaggccgggcgaccaaaggtcgcccgacgcccgggctttgcccgggcggcctcagtgagcgagcgagcgcgcagagagggagtggccaactccatcactaggggttcctagatctgaattcggtaccccactacgggtttaggctgcccatgtaaggaggcaaggcctggggacacccgagatgcctggttataattaacccagacatgtggctgccccccccccccccaacacctgctgcctctaaaaataaccctgtccctggtggatcccctgcatgcgaagatcttcgaacaaggctgtgggggactgagggcaggctgtaacaggcttgggggccagggcttatacgtgcctgggactcccaaagtattactgttccatgttcccggcgaagggccagctgtcccccgccagctagactcagcacttagtttaggaaccagtgagcaagtcagcccttggggcagcccatacaaggccatggggctgggcaagctgcacgcctgggtccggggtgggcacggtgcccgggcaacgagctgaaagctcatctgctctcaggggcccctccctggggacagcccctcctggctagtcacaccctgtaggctcctctatataacccaggggcacaggggctgccctcattctaccaccacctccacagcacagacagacactcaggagccagccagcgtcgagcggccgatccgccaccatgctttggtgggaggaagtggaggactgctacgagagagaggacgtgcagaagaaaaccttcaccaagtgggtgaacgcccagttcagcaagttcggcaagcagcacatcgagaacctgttcagcgacctgcaggatggcaggagactgctggacctgctggagggcctgaccggccagaagctgcccaaggagaagggcagcaccagagtgcacgccctgaacaacgtgaacaaggccctgagagtgctgcagaacaacaacgtggacctggtgaacatcggcagcaccgacatcgtggacggcaaccacaagctgaccctgggcctgatctggaacatcatcctgcactggcaggtgaagaacgtgatgaagaacatcatggccggcctgcagcagaccaacagcgagaagatcctgctgagctgggtgaggcagagcaccagaaactacccccaggtgaacgtgatcaacttcaccacctcctggagcgacggcctggccctgaacgccctgatccacagccacagacccgacctgttcgactggaacagcgtggtgtgtcagcagagcgccacccagagactggagcacgccttcaacatcgccagataccagctgggcatcgagaagctgctggaccccgaggacgtggacaccacctaccccgacaagaaaagcatcctcatgtacattaccagcctgttccaggtgctgccccagcaggtgtccatcgaggccatccaggaagtggaaatgctgcccaggccccccaaagtgaccaaggaggagcacttccagctgcaccaccagatgcactacagccagcagatcacagtgagcctggcccagggctatgagagaaccagcagccccaagcccagattcaagagctacgcctacacccaggccgcctacgtgaccacctccgaccccaccagaagccccttccccagccagcacctggaggcccccgaggacaagagcttcggcagcagcctgatggagagcgaagtgaacctggacagataccagaccgccctggaggaagtgctgtcctggctgctgagcgccgaggacaccctgcaggcccagggcgagatcagcaacgacgtggaagtggtgaaggaccagttccacacccacgagggctacatgatggatctgaccgcccaccagggcagagtgggcaatatcctgcagctgggcagcaagctgatcggcaccggcaagctgagcgaggacgaggagaccgaagtgcaggagcagatgaacctgctgaacagcagatgggagtgcctgagagtggccagcatggagaagcagagcaacctgcacagagtgctgatggacctgcagaaccagaagctgaaggagctgaacgactggctgaccaagaccgaggagcggaccagaaagatggaggaggagcccctgggccccgacctggaggacctgaagagacaggtgcagcagcacaaagtgctgcaggaggacctggagcaggagcaggtgcgcgtgaacagcctgacccacatggtggtggtcgtggacgagagcagcggcgaccacgccacagccgccctggaagagcagctgaaagtgctgggcgacagatgggccaatatttgtaggtggaccgaggacagatgggtgctgctgcaggaccagcccgacctggcccctggcctgaccaccatcggcgccagccccacccagaccgtgaccctggtgacccagcccgtggtgacaaaggagaccgccatcagcaagctggagatgcccagctccctgatgctggaagtgcccacccaccgcctgctccagcagttccccctggacctggagaagttcctggcctggctgaccgaggccgaaaccaccgccaatgtgctccaggacgccactagaaaggagaggctgctggaggacagcaagggcgtgaaagagctgatgaagcagtggcaggatctgcagggcgaaatcgaggcccacaccgacgtgtaccacaacctggacgagaacagccagaagattctgaggagcctggagggcagcgacgacgccgtcctgctccagaggaggctggacaacatgaacttcaagtggagcgagctgcggaagaagagcctgaacatccggagccacctggaagccagcagcgaccagtggaagagactgcacctgagcctgcaggagctgctggtgtggctgcagctgaaggacgacgagctgagcagacaggcccccatcggcggcgacttccccgccgtgcagaagcagaacgacgtgcaccgggccttcaagagggagctgaaaaccaaggaacccgtgatcatgagcaccctggagacagtgcggatcttcctgaccgagcagcccctggagggactggagaagctgtaccaggagcccagagagctgccccccgaggagagagcccagaacgtgaccaggctgctgagaaagcaggccgaggaagtgaataccgagtgggagaagctgaatctgcacagcgccgactggcagagaaagatcgacgagaccctggagagactccaggaactgcaggaagccaccgacgagctggacctgaagctgagacaggccgaagtgatcaagggcagctggcagcctgtgggcgatctgctgatcgactccctgcaggatcacctggagaaagtgaaggccctgcggggcgagatcgcccccctgaaggagaatgtgagccacgtgaacgacctggccagacagctgaccaccctgggcatccagctgagcccctacaacctgagcacactggaggatctgaacacccggtggaaactgctgcaggtggccgtggaggatagagtgaggcagctgcacgaagcccacagagacttcggccctgcctcccagcacttcctgagcaccagcgtgcagggcccctgggagagagccatctcccccaacaaagtgccctactacatcaaccacgagacccagaccacctgctgggaccaccctaagatgaccgagctgtatcagagcctggccgacctgaacaatgtgcggttcagcgcctacagaaccgccatgaagctgcggagactgcagaaggccctgtgcctggatctgctgagcctgagcgccgcctgcgacgccctggaccagcacaacctgaagcagaatgaccagcccatggacatcctgcagatcatcaactgcctgaccacaatctacgaccggctggaacaggagcacaacaacctggtgaatgtgcccctgtgcgtggacatgtgcctgaattggctgctgaacgtgtacgacaccggcaggaccggcagaatccgcgtgctgagcttcaagaccggcatcatcagcctgtgcaaggcccacctggaggataagtaccgctacctgttcaagcaggtggccagcagcaccggcttctgcgatcagaggagactgggcctgctgctgcacgatagcatccagatccctaggcagctgggcgaagtggccagctttggcggcagcaacatcgagccctctgtgaggagctgcttccagttcgccaacaacaagcccgagatcgaggccgccctgttcctggactggatgaggctggagcctcagagcatggtgtggctgcctgtgctgcacagagtggccgccgccgagaccgccaagcaccaggccaagtgcaatatctgcaaggagtgccccatcatcggcttccggtacaggagcctgaagcacttcaactacgacatctgccagagctgctttttcagcggcagagtggccaagggccacaaaatgcactaccccatggtggagtactgcacccccaccacctccggcgaggatgtgagagacttcgccaaagtgctgaagaataagttccggaccaagcggtactttgccaagcaccccaggatgggctacctgcccgtgcagaccgtgctggaaggcgacaacatggagacctgatgaggagctcgagaggcctaataaagagctcagatgcatcgatcagagtgtgttggttttttgtgtgagatctaggaacccctagtgatggagttggccactccctctctgcgcgctcgctcgctcactgaggccgcccgggcaaagcccgggcgtcgggcgacctttggtcgcccggcctcagtgagcgagcgagcgcgcagagagggagtggccaa

SEQ ID NO: 10 - DNA, 4812 bp, Artificial Sequence
  AAV vector genome with Hopti-Dys3837 gene
ttggccactccctctctgcgcgctcgctcgctcactgaggccgggcgaccaaaggtcgcccgacgcccgggctttgcccgggcggcctcagtgagcgagcgagcgcgcagagagggagtggccaactccatcactaggggttcctagatctgaattcggtaccccactacgggtttaggctgcccatgtaaggaggcaaggcctggggacacccgagatgcctggttataattaacccagacatgtggctgccccccccccccccaacacctgctgcctctaaaaataaccctgtccctggtggatcccctgcatgcgaagatcttcgaacaaggctgtgggggactgagggcaggctgtaacaggcttgggggccagggcttatacgtgcctgggactcccaaagtattactgttccatgttcccggcgaagggccagctgtcccccgccagctagactcagcacttagtttaggaaccagtgagcaagtcagcccttggggcagcccatacaaggccatggggctgggcaagctgcacgcctgggtccggggtgggcacggtgcccgggcaacgagctgaaagctcatctgctctcaggggcccctccctggggacagcccctcctggctagtcacaccctgtaggctcctctatataacccaggggcacaggggctgccctcattctaccaccacctccacagcacagacagacactcaggagccagccagcgtcgagcggccgatccgccaccatgctttggtgggaggaagtggaggactgctacgagagagaggacgtgcagaagaaaaccttcaccaagtgggtgaacgcccagttcagcaagttcggcaagcagcacatcgagaacctgttcagcgacctgcaggatggcaggagactgctggacctgctggagggcctgaccggccagaagctgcccaaggagaagggcagcaccagagtgcacgccctgaacaacgtgaacaaggccctgagagtgctgcagaacaacaacgtggacctggtgaacatcggcagcaccgacatcgtggacggcaaccacaagctgaccctgggcctgatctggaacatcatcctgcactggcaggtgaagaacgtgatgaagaacatcatggccggcctgcagcagaccaacagcgagaagatcctgctgagctgggtgaggcagagcaccagaaactacccccaggtgaacgtgatcaacttcaccacctcctggagcgacggcctggccctgaacgccctgatccacagccacagacccgacctgttcgactggaacagcgtggtgtgtcagcagagcgccacccagagactggagcacgccttcaacatcgccagataccagctgggcatcgagaagctgctggaccccgaggacgtggacaccacctaccccgacaagaaaagcatcctcatgtacattaccagcctgttccaggtgctgccccagcaggtgtccatcgaggccatccaggaagtggaaatgctgcccaggccccccaaagtgaccaaggaggagcacttccagctgcaccaccagatgcactacagccagcagatcacagtgagcctggcccagggctatgagagaaccagcagccccaagcccagattcaagagctacgcctacacccaggccgcctacgtgaccacctccgaccccaccagaagccccttccccagccagcacctggaggcccccgaggacaagagcttcggcagcagcctgatggagagcgaagtgaacctggacagataccagaccgccctggaggaagtgctgtcctggctgctgagcgccgaggacaccctgcaggcccagggcgagatcagcaacgacgtggaagtggtgaaggaccagttccacacccacgagggctacatgatggatctgaccgcccaccagggcagagtgggcaatatcctgcagctgggcagcaagctgatcggcaccggcaagctgagcgaggacgaggagaccgaagtgcaggagcagatgaacctgctgaacagcagatgggagtgcctgagagtggccagcatggagaagcagagcaacctgcacagagtgctgatggacctgcagaaccagaagctgaaggagctgaacgactggctgaccaagaccgaggagcggaccagaaagatggaggaggagcccctgggccccgacctggaggacctgaagagacaggtgcagcagcacaaagtgctgcaggaggacctggagcaggagcaggtgcgcgtgaacagcctgacccacatggtggtggtcgtggacgagagcagcggcgaccacgccacagccgccctggaagagcagctgaaagtgctgggcgacagatgggccaatatttgtaggtggaccgaggacagatgggtgctgctgcaggacacccaccgcctgctccagcagttccccctggacctggagaagttcctggcctggctgaccgaggccgaaaccaccgccaatgtgctccaggacgccactagaaaggagaggctgctggaggacagcaagggcgtgaaagagctgatgaagcagtggcaggatctgcagggcgaaatcgaggcccacaccgacgtgtaccacaacctggacgagaacagccagaagattctgaggagcctggagggcagcgacgacgccgtcctgctccagaggaggctggacaacatgaacttcaagtggagcgagctgcggaagaagagcctgaacatccggagccacctggaagccagcagcgaccagtggaagagactgcacctgagcctgcaggagctgctggtgtggctgcagctgaaggacgacgagctgagcagacaggcccccatcggcggcgacttccccgccgtgcagaagcagaacgacgtgcaccgggccttcaagagggagctgaaaaccaaggaacccgtgatcatgagcaccctggagacagtgcggatcttcctgaccgagcagcccctggagggactggagaagctgtaccaggagcccagagagctgccccccgaggagagagcccagaacgtgaccaggctgctgagaaagcaggccgaggaagtgaataccgagtgggagaagctgaatctgcacagcgccgactggcagagaaagatcgacgagaccctggagagactccaggaactgcaggaagccaccgacgagctggacctgaagctgagacaggccgaagtgatcaagggcagctggcagcctgtgggcgatctgctgatcgactccctgcaggatcacctggagaaagtgaaggccctgcggggcgagatcgcccccctgaaggagaatgtgagccacgtgaacgacctggccagacagctgaccaccctgggcatccagctgagcccctacaacctgagcacactggaggatctgaacacccggtggaaactgctgcaggtggccgtggaggatagagtgaggcagctgcacgaagcccacagagacttcggccctgcctcccagcacttcctgagcaccagcgtgcagggcccctgggagagagccatctcccccaacaaagtgccctactacatcaaccacgagacccagaccacctgctgggaccaccctaagatgaccgagctgtatcagagcctggccgacctgaacaatgtgcggttcagcgcctacagaaccgccatgaagctgcggagactgcagaaggccctgtgcctggatctgctgagcctgagcgccgcctgcgacgccctggaccagcacaacctgaagcagaatgaccagcccatggacatcctgcagatcatcaactgcctgaccacaatctacgaccggctggaacaggagcacaacaacctggtgaatgtgcccctgtgcgtggacatgtgcctgaattggctgctgaacgtgtacgacaccggcaggaccggcagaatccgcgtgctgagcttcaagaccggcatcatcagcctgtgcaaggcccacctggaggataagtaccgctacctgttcaagcaggtggccagcagcaccggcttctgcgatcagaggagactgggcctgctgctgcacgatagcatccagatccctaggcagctgggcgaagtggccagctttggcggcagcaacatcgagccctctgtgaggagctgcttccagttcgccaacaacaagcccgagatcgaggccgccctgttcctggactggatgaggctggagcctcagagcatggtgtggctgcctgtgctgcacagagtggccgccgccgagaccgccaagcaccaggccaagtgcaatatctgcaaggagtgccccatcatcggcttccggtacaggagcctgaagcacttcaactacgacatctgccagagctgctttttcagcggcagagtggccaagggccacaaaatgcactaccccatggtggagtactgcacccccaccacctccggcgaggatgtgagagacttcgccaaagtgctgaagaataagttccggaccaagcggtactttgccaagcaccccaggatgggctacctgcccgtgcagaccgtgctggaaggcgacaacatggagacctgatgaggagctcgagaggcctaataaagagctcagatgcatcgatcagagtgtgttggttttttgtgtgagatctaggaacccctagtgatggagttggccactccctctctgcgcgctcgctcgctcactgaggccgcccgggcaaagcccgggcgtcgggcgacctttggtcgcccggcctcagtgagcgagcgagcgcgcagagagggagtggccaa

SEQ ID NO: 11 - DNA, 4965 bp, Artificial Sequence
  AAV vector genome with Hopti-Dys3837 gene
ttggccactccctctctgcgcgctcgctcgctcactgaggccgggcgaccaaaggtcgcccgacgcccgggctttgcccgggcggcctcagtgagcgagcgagcgcgcagagagggagtggccaactccatcactaggggttcctagatctgaattcggtaccccactacgggtctaggctgcccatgtaaggaggcaaggcctggggacacccgagatgcctggttataattaaccccaacacctgctgcccccccccccccaacacctgctgcctctaaaaataaccctgtccctggtggatcccctgcatgccccactacgggtttaggctgcccatgtaaggaggcaaggcctggggacacccgagatgcctggttataattaacccagacatgtggctgccccccccccccccaacacctgctgcctctaaaaataaccctgtccctggtggatcccctgcatgcgaagatcttcgaacaaggctgtgggggactgagggcaggctgtaacaggcttgggggccagggcttatacgtgcctgggactcccaaagtattactgttccatgttcccggcgaagggccagctgtcccccgccagctagactcagcacttagtttaggaaccagtgagcaagtcagcccttggggcagcccatacaaggccatggggctgggcaagctgcacgcctgggtccggggtgggcacggtgcccgggcaacgagctgaaagctcatctgctctcaggggcccctccctggggacagcccctcctggctagtcacaccctgtaggctcctctatataacccaggggcacaggggctgccctcattctaccaccacctccacagcacagacagacactcaggagccagccagcgtcgagcggccgatccgccaccatgctttggtgggaggaagtggaggactgctacgagagagaggacgtgcagaagaaaaccttcaccaagtgggtgaacgcccagttcagcaagttcggcaagcagcacatcgagaacctgttcagcgacctgcaggatggcaggagactgctggacctgctggagggcctgaccggccagaagctgcccaaggagaagggcagcaccagagtgcacgccctgaacaacgtgaacaaggccctgagagtgctgcagaacaacaacgtggacctggtgaacatcggcagcaccgacatcgtggacggcaaccacaagctgaccctgggcctgatctggaacatcatcctgcactggcaggtgaagaacgtgatgaagaacatcatggccggcctgcagcagaccaacagcgagaagatcctgctgagctgggtgaggcagagcaccagaaactacccccaggtgaacgtgatcaacttcaccacctcctggagcgacggcctggccctgaacgccctgatccacagccacagacccgacctgttcgactggaacagcgtggtgtgtcagcagagcgccacccagagactggagcacgccttcaacatcgccagataccagctgggcatcgagaagctgctggaccccgaggacgtggacaccacctaccccgacaagaaaagcatcctcatgtacattaccagcctgttccaggtgctgccccagcaggtgtccatcgaggccatccaggaagtggaaatgctgcccaggccccccaaagtgaccaaggaggagcacttccagctgcaccaccagatgcactacagccagcagatcacagtgagcctggcccagggctatgagagaaccagcagccccaagcccagattcaagagctacgcctacacccaggccgcctacgtgaccacctccgaccccaccagaagccccttccccagccagcacctggaggcccccgaggacaagagcttcggcagcagcctgatggagagcgaagtgaacctggacagataccagaccgccctggaggaagtgctgtcctggctgctgagcgccgaggacaccctgcaggcccagggcgagatcagcaacgacgtggaagtggtgaaggaccagttccacacccacgagggctacatgatggatctgaccgcccaccagggcagagtgggcaatatcctgcagctgggcagcaagctgatcggcaccggcaagctgagcgaggacgaggagaccgaagtgcaggagcagatgaacctgctgaacagcagatgggagtgcctgagagtggccagcatggagaagcagagcaacctgcacagagtgctgatggacctgcagaaccagaagctgaaggagctgaacgactggctgaccaagaccgaggagcggaccagaaagatggaggaggagcccctgggccccgacctggaggacctgaagagacaggtgcagcagcacaaagtgctgcaggaggacctggagcaggagcaggtgcgcgtgaacagcctgacccacatggtggtggtcgtggacgagagcagcggcgaccacgccacagccgccctggaagagcagctgaaagtgctgggcgacagatgggccaatatttgtaggtggaccgaggacagatgggtgctgctgcaggacacccaccgcctgctccagcagttccccctggacctggagaagttcctggcctggctgaccgaggccgaaaccaccgccaatgtgctccaggacgccactagaaaggagaggctgctggaggacagcaagggcgtgaaagagctgatgaagcagtggcaggatctgcagggcgaaatcgaggcccacaccgacgtgtaccacaacctggacgagaacagccagaagattctgaggagcctggagggcagcgacgacgccgtcctgctccagaggaggctggacaacatgaacttcaagtggagcgagctgcggaagaagagcctgaacatccggagccacctggaagccagcagcgaccagtggaagagactgcacctgagcctgcaggagctgctggtgtggctgcagctgaaggacgacgagctgagcagacaggcccccatcggcggcgacttccccgccgtgcagaagcagaacgacgtgcaccgggccttcaagagggagctgaaaaccaaggaacccgtgatcatgagcaccctggagacagtgcggatcttcctgaccgagcagcccctggagggactggagaagctgtaccaggagcccagagagctgccccccgaggagagagcccagaacgtgaccaggctgctgagaaagcaggccgaggaagtgaataccgagtgggagaagctgaatctgcacagcgccgactggcagagaaagatcgacgagaccctggagagactccaggaactgcaggaagccaccgacgagctggacctgaagctgagacaggccgaagtgatcaagggcagctggcagcctgtgggcgatctgctgatcgactccctgcaggatcacctggagaaagtgaaggccctgcggggcgagatcgcccccctgaaggagaatgtgagccacgtgaacgacctggccagacagctgaccaccctgggcatccagctgagcccctacaacctgagcacactggaggatctgaacacccggtggaaactgctgcaggtggccgtggaggatagagtgaggcagctgcacgaagcccacagagacttcggccctgcctcccagcacttcctgagcaccagcgtgcagggcccctgggagagagccatctcccccaacaaagtgccctactacatcaaccacgagacccagaccacctgctgggaccaccctaagatgaccgagctgtatcagagcctggccgacctgaacaatgtgcggttcagcgcctacagaaccgccatgaagctgcggagactgcagaaggccctgtgcctggatctgctgagcctgagcgccgcctgcgacgccctggaccagcacaacctgaagcagaatgaccagcccatggacatcctgcagatcatcaactgcctgaccacaatctacgaccggctggaacaggagcacaacaacctggtgaatgtgcccctgtgcgtggacatgtgcctgaattggctgctgaacgtgtacgacaccggcaggaccggcagaatccgcgtgctgagcttcaagaccggcatcatcagcctgtgcaaggcccacctggaggataagtaccgctacctgttcaagcaggtggccagcagcaccggcttctgcgatcagaggagactgggcctgctgctgcacgatagcatccagatccctaggcagctgggcgaagtggccagctttggcggcagcaacatcgagccctctgtgaggagctgcttccagttcgccaacaacaagcccgagatcgaggccgccctgttcctggactggatgaggctggagcctcagagcatggtgtggctgcctgtgctgcacagagtggccgccgccgagaccgccaagcaccaggccaagtgcaatatctgcaaggagtgccccatcatcggcttccggtacaggagcctgaagcacttcaactacgacatctgccagagctgctttttcagcggcagagtggccaagggccacaaaatgcactaccccatggtggagtactgcacccccaccacctccggcgaggatgtgagagacttcgccaaagtgctgaagaataagttccggaccaagcggtactttgccaagcaccccaggatgggctacctgcccgtgcagaccgtgctggaaggcgacaacatggagacctgatgaggagctcgagaggcctaataaagagctcagatgcatcgatcagagtgtgttggttttttgtgtgagatctaggaacccctagtgatggagttggccactccctctctgcgcgctcgctcgctcactgaggccgcccgggcaaagcccgggcgtcgggcgacctttggtcgcccggcctcagtgagcgagcgagcgcgcagagagggagtggccaa

SEQ ID NO: 12 - DNA, 4955 bp, Artificial Sequence
  AAV vector genome with Copti-Dys3978 gene
ttggccactccctctctgcgcgctcgctcgctcactgaggccgggcgaccaaaggtcgcccgacgcccgggctttgcccgggcggcctcagtgagcgagcgagcgcgcagagagggagtggccaactccatcactaggggttcctcagatctgaattcggtaccccactacgggtttaggctgcccatgtaaggaggcaaggcctggggacacccgagatgcctggttataattaacccagacatgtggctgccccccccccccccaacacctgctgcctctaaaaataaccctgtccctggtggatcccctgcatgcgaagatcttcgaacaaggctgtgggggactgagggcaggctgtaacaggcttgggggccagggcttatacgtgcctgggactcccaaagtattactgttccatgttcccggcgaagggccagctgtcccccgccagctagactcagcacttagtttaggaaccagtgagcaagtcagcccttggggcagcccatacaaggccatggggctgggcaagctgcacgcctgggtccggggtgggcacggtgcccgggcaacgagctgaaagctcatctgctctcaggggcccctccctggggacagcccctcctggctagtcacaccctgtaggctcctctatataacccaggggcacaggggctgccctcattctaccaccacctccacagcacagacagacactcaggagccagccagcgtcgagcggccgccaccatgctttggtgggaggaagtggaggactgctacgagcgggaggacgtgcagaagaaaaccttcaccaagtgggtgaacgcccagttcagcaagttcggcaagcagcacatcgagaacctgttcagcgacctgcaggacggcaggcggctgctggacctcctggaaggcctgaccggccagaagctgcccaaagagaagggcagcaccagggtgcacgccctgaacaacgtgaacaaggccctgagggtgctgcagaacaacaacgtggacctggtgaacatcggcagcaccgacatcgtggacggcaaccacaagctgaccctgggcctgatctggaacatcatcctgcactggcaggtcaagaacgtgatgaagaacatcatggccggcctgcagcagaccaacagcgagaagatcctgctgtcctgggtgcggcagagcaccaggaactacccccaggtcaacgtgatcaacttcaccacctcttggagcgacggcctggccctgaacgccctgatccacagccacaggcccgacctgttcgactggaacagcgtggtgtgccagcagagcgccacccagaggctggaacacgccttcaacatcgccagataccagctgggcatcgagaagctgctggatcccgaggacgtggacaccacctaccccgacaagaaaagcatcctcatgtacatcaccagcctgttccaggtgctgccccagcaggtgtccatcgaggccatccaggaagtggagatgctgcccaggccccccaaggtcaccaaagaggaacacttccagctgcaccaccagatgcactacagccagcagatcaccgtgagcctggcccagggctacgagaggaccagcagccccaagcccaggttcaagagctacgcctacacccaggccgcctacgtgaccacctccgaccccaccaggtcccccttccccagccagcatctcgaagcccccgaggacaagagcttcggcagcagcctgatggaaagcgaggtgaacctggacagataccagaccgccctggaagaagtgctgtcttggctgctgtccgccgaggacaccctgcaggcccagggcgagatcagcaacgacgtggaggtcgtgaaggaccagttccacacccacgagggctacatgatggacctgaccgcccaccagggcagagtgggcaacatcctgcagctgggcagcaagctgatcggcaccggcaagctgtccgaggacgaggaaaccgaggtgcaggaacagatgaacctgctgaacagcagatgggagtgcctgagggtggccagcatggaaaagcagagcaacctgcacagggtgctgatggatctgcagaaccagaagctcaaagagctgaacgactggctgaccaagaccgaggaaaggacccggaagatggaagaggaacccctgggccccgatctcgaagatctgaagaggcaggtgcagcagcacaaggtgctgcaggaagatctcgaacaggaacaggtccgggtcaacagcctgacccacatggtcgtggtggtggacgagagcagcggcgaccacgccaccgctgccctggaagagcagctgaaggtgctgggcgacagatgggccaacatctgccggtggaccgaggacagatgggtcctcctgcaggaccagcccgacctggcccctggcctgacaaccatcggcgccagccccacccagaccgtgaccctggtgacccagcccgtggtgaccaaagagaccgccatcagcaagctggaaatgcccagctccctgatgctggaagtgcccacccacaggctcctccagcagttccccctggacctggaaaagttcctggcctggctgaccgaggccgagaccaccgccaacgtgctgcaggacgccaccaggaaagagaggctgctggaagatagcaagggcgtgaaagagctgatgaagcagtggcaggacctgcagggggagattgaggcccacaccgacgtgtaccacaacctggacgagaacagccagaaaatcctgagaagcctggaaggcagcgacgacgccgtgctgctgcagaggcggctggacaacatgaacttcaagtggagcgagctgaggaagaagagcctgaacatcaggtcccatctggaagccagcagcgaccagtggaagaggctgcacctgagcctgcaggaactgctcgtctggctgcagctgaaagacgacgagctgtccaggcaggcccccatcggcggcgacttccccgccgtgcagaaacagaacgacgtgcacagggccttcaagcgggagctgaaaaccaaagagcccgtgatcatgagcaccctggaaaccgtgaggatcttcctgaccgagcagcccctggaaggactggaaaagctgtaccaggaacccagagagctgccccccgaggaacgggcccagaacgtgaccaggctgctgagaaagcaggccgaggaagtgaacaccgagtgggagaagctgaacctgcactccgccgactggcagaggaagatcgacgagaccctggaaaggctccaggaactgcaggaagccaccgacgagctggacctgaagctgagacaggccgaggtgatcaagggcagctggcagcccgtgggcgacctgctgatcgactccctgcaggatcacctggaaaaagtgaaggccctgcggggcgagatcgcccccctgaaagagaacgtcagccacgtcaacgacctggccaggcagctgaccaccctgggcatccagctgtccccctacaacctgtccaccctggaagatctgaacacaaggtggaagctgctgcaggtggccgtggaggacagagtgaggcagctgcacgaggcccacagggacttcggccctgcctcccagcacttcctgagcaccagcgtgcagggcccctgggagagggccatctcccccaacaaggtgccctactacatcaaccacgagacccagaccacctgctgggaccaccctaagatgaccgagctgtaccagtccctggccgacctgaacaatgtgcggttcagcgcctaccggaccgccatgaagctgaggcggctgcagaaagccctgtgcctggatctgctgtccctgagcgccgcctgcgacgccctggaccagcacaacctgaagcagaacgaccagcccatggatatcctgcagatcatcaactgtctgaccaccatctacgacaggctggaacaggaacacaacaacctggtcaacgtgcccctgtgcgtggacatgtgcctgaactggctgctgaacgtgtacgacaccggcaggaccggccggatcagggtgctgtccttcaagaccggcatcatcagcctgtgcaaggcccacctggaagataagtaccgctacctgttcaagcaggtggccagctctaccggcttctgcgaccagcggaggctgggcctgctgctgcacgacagcatccagatcccccggcagctgggcgaggtggcctccttcggcggcagcaacatcgagcccagcgtgcggagctgcttccagttcgccaacaacaagcccgagatcgaggccgccctgttcctggactggatgcggctggaaccccagagcatggtctggctgcccgtgctgcacagagtggctgccgccgagaccgccaagcaccaggccaagtgcaacatctgcaaagagtgccccatcatcggcttcaggtacagaagcctgaagcacttcaactacgacatctgccagagctgtttcttcagcggcagggtggccaagggccacaaaatgcactaccccatggtggagtactgcacccccaccacctccggcgaggacgtgagggacttcgccaaggtgctgaagaataagttccggaccaagcggtacttcgccaaacaccccaggatgggctacctgcccgtgcagaccgtgctggaaggcgacaacatggaaacctgataacacgcgtcgactcgagaggcctaataaagagctcagatgcatcgatcagagtgtgttggttttttgtgtgagatctaggaacccctagtgatggagttggccactccctctctgcgcgctcgctcgctcactgaggccgcccgggcaaagcccgggcgtcgggcgacctttggtcgcccggcctcagtgagcgagcgagcgcgcagagagggagtggccaa

SEQ ID NO: 13 - protein, 736 aa, adeno-associated virus 9
MAADGYLPDWLEDNLSEGIREWWALKPGAPQPKANQQHQDNARGLVLPGYKYLGPGNGLDKGEPVNAADAAALEHDKAYDQQLKAGDNPYLKYNHADAEFQERLKEDTSFGGNLGRAVFQAKKRLLEPLGLVEEAAKTAPGKKRPVEQSPQEPDSSAGIGKSGAQPAKKRLNFGQTGDTESVPDPQPIGEPPAAPSGVGSLTMASGGGAPVADNNEGADGVGSSSGNWHCDSQWLGDRVITTSTRTWALPTYNNHLYKQISNSTSGGSSNDNAYFGYSTPWGYFDFNRFHCHFSPRDWQRLINNNWGFRPKRLNFKLFNIQVKEVTDNNGVKTIANNLTSTVQVFTDSDYQLPYVLGSAHEGCLPPFPADVFMIPQYGYLTLNDGSQAVGRSSFYCLEYFPSQMLRTGNNFQFSYEFENVPFHSSYAHSQSLDRLMNPLIDQYLYYLSKTINGSGQNQQTLKFSVAGPSNMAVQGRNYIPGPSYRQQRVSTTVTQNNNSEFAWPGASSWALNGRNSLMNPGPAMASHKEGEDRFFPLSGSLIFGKQGTGRDNVDADKVMITNEEEIKTTNPVATESYGQVATNHQSAQAQAQTGWVQNQGILPGMVWQDRDVYLQGPIWAKIPHTDGNFHPSPLMGGFGMKHPPPQILIKNTPVPADPPTAFNKDKLNSFITQYSTGQVSVEIEWELQKENSKRWNPEIQYTSNYYKSNNVEFAVNTEGVYSEPRPIGTRYLTRNL

SEQ ID NO: 14 - DNA, 145 bp, adeno-associated virus 2
ttggccactccctctctgcgcgctcgctcgctcactgaggccgggcgaccaaaggtcgcccgacgcccgggctttgcccgggcggcctcagtgagcgagcgagcgcgcagagagggagtggccaactccatcactaggggttcct

SEQ ID NO: 15 - DNA, 145 bp, adeno-associated virus 2
aggaacccctagtgatggagttggccactccctctctgcgcgctcgctcgctcactgaggccgcccgggcaaagcccgggcgtcgggcgacctttggtcgcccggcctcagtgagcgagcgagcgcgcagagagggagtggccaa

SEQ ID NO: 16 - DNA, 577 bp, Artificial Sequence
  Synthetic enhancer and promoter
ccactacgggtctaggctgcccatgtaaggaggcaaggcctggggacacccgagatgcctggttataattaacccagacatgtggctgccccccccccccccaacacctgctgcctctaaaaataaccctgtccctggtggatcccctgcatgcgaagatcttcgaacaaggctgtgggggactgagggcaggctgtaacaggcttgggggccagggcttatacgtgcctgggactcccaaagtattactgttccatgttcccggcgaagggccagctgtcccccgccagctagactcagcacttagtttaggaaccagtgagcaagtcagcccttggggcagcccatacaaggccatggggctgggcaagctgcacgcctgggtccggggtgggcacggtgcccgggcaacgagctgaaagctcatctgctctcaggggcccctccctggggacagcccctcctggctagtcacaccctgtaggctcctctatataacccaggggcacaggggctgccctcattctaccaccacctccacagcacagacagacactcaggagccagccagcgtcga

SEQ ID NO: 17 - DNA, 54 bp, Artificial Sequence
  Synthetic transcription terminator
aggcctaataaagagctcagatgcatcgatcagagtgtgttggttttttgtgtg

SEQ ID NO: 18 - DNA, 4955 bp, Artificial Sequence
  AAV vector genome with Hopti-Dys3978 gene
ttggccactccctctctgcgcgctcgctcgctcactgaggccgggcgaccaaaggtcgcccgacgcccgggctttgcccgggcggcctcagtgagcgagcgagcgcgcagagagggagtggccaactccatcactaggggttcctcagatctgaattcggtaccccactacgggtctaggctgcccatgtaaggaggcaaggcctggggacacccgagatgcctggttataattaacccagacatgtggctgccccccccccccccaacacctgctgcctctaaaaataaccctgtccctggtggatcccctgcatgcgaagatcttcgaacaaggctgtgggggactgagggcaggctgtaacaggcttgggggccagggcttatacgtgcctgggactcccaaagtattactgttccatgttcccggcgaagggccagctgtcccccgccagctagactcagcacttagtttaggaaccagtgagcaagtcagcccttggggcagcccatacaaggccatggggctgggcaagctgcacgcctgggtccggggtgggcacggtgcccgggcaacgagctgaaagctcatctgctctcaggggcccctccctggggacagcccctcctggctagtcacaccctgtaggctcctctatataacccaggggcacaggggctgccctcattctaccaccacctccacagcacagacagacactcaggagccagccagcgtcgagcggccgatccgccaccatgctttggtgggaggaagtggaggactgctacgagagagaggacgtgcagaagaaaaccttcaccaagtgggtgaacgcccagttcagcaagttcggcaagcagcacatcgagaacctgttcagcgacctgcaggatggcaggagactgctggacctgctggagggcctgaccggccagaagctgcccaaggagaagggcagcaccagagtgcacgccctgaacaacgtgaacaaggccctgagagtgctgcagaacaacaacgtggacctggtgaacatcggcagcaccgacatcgtggacggcaaccacaagctgaccctgggcctgatctggaacatcatcctgcactggcaggtgaagaacgtgatgaagaacatcatggccggcctgcagcagaccaacagcgagaagatcctgctgagctgggtgaggcagagcaccagaaactacccccaggtgaacgtgatcaacttcaccacctcctggagcgacggcctggccctgaacgccctgatccacagccacagacccgacctgttcgactggaacagcgtggtgtgtcagcagagcgccacccagagactggagcacgccttcaacatcgccagataccagctgggcatcgagaagctgctggaccccgaggacgtggacaccacctaccccgacaagaaaagcatcctcatgtacattaccagcctgttccaggtgctgccccagcaggtgtccatcgaggccatccaggaagtggaaatgctgcccaggccccccaaagtgaccaaggaggagcacttccagctgcaccaccagatgcactacagccagcagatcacagtgagcctggcccagggctatgagagaaccagcagccccaagcccagattcaagagctacgcctacacccaggccgcctacgtgaccacctccgaccccaccagaagccccttccccagccagcacctggaggcccccgaggacaagagcttcggcagcagcctgatggagagcgaagtgaacctggacagataccagaccgccctggaggaagtgctgtcctggctgctgagcgccgaggacaccctgcaggcccagggcgagatcagcaacgacgtggaagtggtgaaggaccagttccacacccacgagggctacatgatggatctgaccgcccaccagggcagagtgggcaatatcctgcagctgggcagcaagctgatcggcaccggcaagctgagcgaggacgaggagaccgaagtgcaggagcagatgaacctgctgaacagcagatgggagtgcctgagagtggccagcatggagaagcagagcaacctgcacagagtgctgatggacctgcagaaccagaagctgaaggagctgaacgactggctgaccaagaccgaggagcggaccagaaagatggaggaggagcccctgggccccgacctggaggacctgaagagacaggtgcagcagcacaaagtgctgcaggaggacctggagcaggagcaggtgcgcgtgaacagcctgacccacatggtggtggtcgtggacgagagcagcggcgaccacgccacagccgccctggaagagcagctgaaagtgctgggcgacagatgggccaatatttgtaggtggaccgaggacagatgggtgctgctgcaggaccagcccgacctggcccctggcctgaccaccatcggcgccagccccacccagaccgtgaccctggtgacccagcccgtggtgacaaaggagaccgccatcagcaagctggagatgcccagctccctgatgctggaagtgcccacccaccgcctgctccagcagttccccctggacctggagaagttcctggcctggctgaccgaggccgaaaccaccgccaatgtgctccaggacgccactagaaaggagaggctgctggaggacagcaagggcgtgaaagagctgatgaagcagtggcaggatctgcagggcgaaatcgaggcccacaccgacgtgtaccacaacctggacgagaacagccagaagattctgaggagcctggagggcagcgacgacgccgtcctgctccagaggaggctggacaacatgaacttcaagtggagcgagctgcggaagaagagcctgaacatccggagccacctggaagccagcagcgaccagtggaagagactgcacctgagcctgcaggagctgctggtgtggctgcagctgaaggacgacgagctgagcagacaggcccccatcggcggcgacttccccgccgtgcagaagcagaacgacgtgcaccgggccttcaagagggagctgaaaaccaaggaacccgtgatcatgagcaccctggagacagtgcggatcttcctgaccgagcagcccctggagggactggagaagctgtaccaggagcccagagagctgccccccgaggagagagcccagaacgtgaccaggctgctgagaaagcaggccgaggaagtgaataccgagtgggagaagctgaatctgcacagcgccgactggcagagaaagatcgacgagaccctggagagactccaggaactgcaggaagccaccgacgagctggacctgaagctgagacaggccgaagtgatcaagggcagctggcagcctgtgggcgatctgctgatcgactccctgcaggatcacctggagaaagtgaaggccctgcggggcgagatcgcccccctgaaggagaatgtgagccacgtgaacgacctggccagacagctgaccaccctgggcatccagctgagcccctacaacctgagcacactggaggatctgaacacccggtggaaactgctgcaggtggccgtggaggatagagtgaggcagctgcacgaagcccacagagacttcggccctgcctcccagcacttcctgagcaccagcgtgcagggcccctgggagagagccatctcccccaacaaagtgccctactacatcaaccacgagacccagaccacctgctgggaccaccctaagatgaccgagctgtatcagagcctggccgacctgaacaatgtgcggttcagcgcctacagaaccgccatgaagctgcggagactgcagaaggccctgtgcctggatctgctgagcctgagcgccgcctgcgacgccctggaccagcacaacctgaagcagaatgaccagcccatggacatcctgcagatcatcaactgcctgaccacaatctacgaccggctggaacaggagcacaacaacctggtgaatgtgcccctgtgcgtggacatgtgcctgaattggctgctgaacgtgtacgacaccggcaggaccggcagaatccgcgtgctgagcttcaagaccggcatcatcagcctgtgcaaggcccacctggaggataagtaccgctacctgttcaagcaggtggccagcagcaccggcttctgcgatcagaggagactgggcctgctgctgcacgatagcatccagatccctaggcagctgggcgaagtggccagctttggcggcagcaacatcgagccctctgtgaggagctgcttccagttcgccaacaacaagcccgagatcgaggccgccctgttcctggactggatgaggctggagcctcagagcatggtgtggctgcctgtgctgcacagagtggccgccgccgagaccgccaagcaccaggccaagtgcaatatctgcaaggagtgccccatcatcggcttccggtacaggagcctgaagcacttcaactacgacatctgccagagctgctttttcagcggcagagtggccaagggccacaaaatgcactaccccatggtggagtactgcacccccaccacctccggcgaggatgtgagagacttcgccaaagtgctgaagaataagttccggaccaagcggtactttgccaagcaccccaggatgggctacctgcccgtgcagaccgtgctggaaggcgacaacatggagacctgatgaggagctcgagaggcctaataaagagctcagatgcatcgatcagagtgtgttggttttttgtgtgagatctgaggaacccctagtgatggagttggccactccctctctgcgcgctcgctcgctcactgaggccgcccgggcaaagcccgggcgtcgggcgacctttggtcgcccggcctcagtgagcgagcgagcgcgcagagagggagtggccaa

SEQ ID NO: 19 - DNA, 23 bp, Artificial Sequence
  Primer
ccaacaaagtgccctactacatc

SEQ ID NO: 20 - DNA, 21 bp, Artificial Sequence
  Primer
ggttgtgctggtccagggcgt

SEQ ID NO: 21 - DNA, 23 bp, Artificial Sequence
  Primer
ccgagctgtatcagagcctggcc

SEQ ID NO: 22 - DNA, 21 bp, Artificial Sequence
  Primer
gcgaaagtggaaaagccaagt

SEQ ID NO: 23 - DNA, 24 bp, Artificial Sequence
  Primer
gccacatcaacaggactcttgtag

SEQ ID NO: 24 - DNA, 30 bp, Artificial Sequence
  Primer
caaagcctaaaagacagcggcaagttgaat

SEQ ID NO: 25 - protein, 3685 aa, Homo sapiens
MLWWEEVEDCYEREDVQKKTFTKWVNAQFSKFGKQHIENLFSDLQDGRRLLDLLEGLTGQKLPKEKGSTRVHALNNVNKALRVLQNNNVDLVNIGSTDIVDGNHKLTLGLIWNIILHWQVKNVMKNIMAGLQQTNSEKILLSWVRQSTRNYPQVNVINFTTSWSDGLALNALIHSHRPDLFDWNSVVCQQSATQRLEHAFNIARYQLGIEKLLDPEDVDTTYPDKKSILMYITSLFQVLPQQVSIEAIQEVEMLPRPPKVTKEEHFQLHHQMHYSQQITVSLAQGYERTSSPKPRFKSYAYTQAAYVTTSDPTRSPFPSQHLEAPEDKSFGSSLMESEVNLDRYQTALEEVLSWLLSAEDTLQAQGEISNDVEVVKDQFHTHEGYMMDLTAHQGRVGNILQLGSKLIGTGKLSEDEETEVQEQMNLLNSRWECLRVASMEKQSNLHRVLMDLQNQKLKELNDWLTKTEERTRKMEEEPLGPDLEDLKRQVQQHKVLQEDLEQEQVRVNSLTHMVVVVDESSGDHATAALEEQLKVLGDRWANICRWTEDRWVLLQDILLKWQRLTEEQCLFSAWLSEKEDAVNKIHTTGFKDQNEMLSSLQKLAVLKADLEKKKQSMGKLYSLKQDLLSTLKNKSVTQKTEAWLDNFARCWDNLVQKLEKSTAQISQAVTTTQPSLTQTTVMETVTTVTTREQILVKHAQEELPPPPPQKKRQITVDSEIRKRLDVDITELHSWITRSEAVLQSPEFAIFRKEGNFSDLKEKVNAIEREKAEKFRKLQDASRSAQALVEQMVNEGVNADSIKQASEQLNSRWIEFCQLLSERLNWLEYQNNIIAFYNQLQQLEQMTTTAENWLKIQPTTPSEPTAIKSQLKICKDEVNRLSGLQPQIERLKIQSIALKEKGQGPMFLDADFVAFTNHFKQVFSDVQAREKELQTIFDTLPPMRYQETMSAIRTWVQQSETKLSIPQLSVTDYEIMEQRLGELQALQSSLQEQQSGLYYLSTTVKEMSKKAPSEISRKYQSEFEEIEGRWKKLSSQLVEHCQKLEEQMNKLRKIQNHIQTLKKWMAEVDVFLKEEWPALGDSEILKKQLKQCRLLVSDIQTIQPSLNSVNEGGQKIKNEAEPEFASRLETELKELNTQWDHMCQQVYARKEALKGGLEKTVSLQKDLSEMHEWMTQAEEEYLERDFEYKTPDELQKAVEEMKRAKEEAQQKEAKVKLLTESVNSVIAQAPPVAQEALKKELETLTTNYQWLCTRLNGKCKTLEEVWACWHELLSYLEKANKWLNEVEFKLKTTENIPGGAEEISEVLDSLENLMRHSEDNPNQIRILAQTLTDGGVMDELINEELETFNSRWRELHEEAVRRQKLLEQSIQSAQETEKSLHLIQESLTFIDKQLAAYIADKVDAAQMPQEAQKIQSDLTSHEISLEEMKKHNQGKEAAQRVLSQIDVAQKKLQDVSMKFRLFQKPANFEQRLQESKMILDEVKMHLPALETKSVEQEVVQSQLNHCVNLYKSLSEVKSEVEMVIKTGRQIVQKKQTENPKELDERVTALKLHYNELGAKVTERKQQLEKCLKLSRKMRKEMNVLTEWLAATDMELTKRSAVEGMPSNLDSEVAWGKATQKEIEKQKVHLKSITEVGEALKTVLGKKETLVEDKLSLLNSNWIAVTSRAEEWLNLLLEYQKHMETFDQNVDHITKWIIQADTLLDESEKKKPQQKEDVLKRLKAELNDIRPKVDSTRDQAANLMANRGDHCRKLVEPQISELNHRFAAISHRIKTGKASIPLKELEQFNSDIQKLLEPLEAEIQQGVNLKEEDFNKDMNEDNEGTVKELLQRGDNLQQRITDERKREEIKIKQQLLQTKHNALKDLRSQRRKKALEISHQWYQYKRQADDLLKCLDDIEKKLASLPEPRDERKIKEIDRELQKKKEELNAVRRQAEGLSEDGAAMAVEPTQIQLSKRWREIESKFAQFRRLNFAQIHTVREETMMVMTEDMPLEISYVPSTYLTEITHVSQALLEVEQLLNAPDLCAKDFEDLFKQEESLKNIKDSLQQSSGRIDIIHSKKTAALQSATPVERVKLQEALSQLDFQWEKVNKMYKDRQGRFDRSVEKWRRFHYDIKIFNQWLTEAEQFLRKTQIPENWEHAKYKWYLKELQDGIGQRQTVVRTLNATGEEIIQQSSKTDASILQEKLGSLNLRWQEVCKQLSDRKKRLEEQKNILSEFQRDLNEFVLWLEEADNIASIPLEPGKEQQLKEKLEQVKLLVEELPLRQGILKQLNETGGPVLVSAPISPEEQDKLENKLKQTNLQWIKVSRALPEKQGEIEAQIKDLGQLEKKLEDLEEQLNHLLLWLSPIRNQLEIYNQPNQEGPFDVQETEIAVQAKQPDVEEILSKGQHLYKEKPATQPVKRKLEDLSSEWKAVNRLLQELRAKQPDLAPGLTTIGASPTQTVTLVTQPVVTKETAISKLEMPSSLMLEVPALADFNRAWTELTDWLSLLDQVIKSQRVMVGDLEDINEMIIKQKATMQDLEQRRPQLEELITAAQNLKNKTSNQEARTIITDRIERIQNQWDEVQEHLQNRRQQLNEMLKDSTQWLEAKEEAEQVLGQARAKLESWKEGPYTVDAIQKKITETKQLAKDLRQWQTNVDVANDLALKLLRDYSADDTRKVHMITENINASWRSIHKRVSEREAALEETHRLLQQFPLDLEKFLAWLTEAETTANVLQDATRKERLLEDSKGVKELMKQWQDLQGEIEAHTDVYHNLDENSQKILRSLEGSDDAVLLQRRLDNMNFKWSELRKKSLNIRSHLEASSDQWKRLHLSLQELLVWLQLKDDELSRQAPIGGDFPAVQKQNDVHRAFKRELKTKEPVIMSTLETVRIFLTEQPLEGLEKLYQEPRELPPEERAQNVTRLLRKQAEEVNTEWEKLNLHSADWQRKIDETLERLQELQEATDELDLKLRQAEVIKGSWQPVGDLLIDSLQDHLEKVKALRGEIAPLKENVSHVNDLARQLTTLGIQLSPYNLSTLEDLNTRWKLLQVAVEDRVRQLHEAHRDFGPASQHFLSTSVQGPWERAISPNKVPYYINHETQTTCWDHPKMTELYQSLADLNNVRFSAYRTAMKLRRLQKALCLDLLSLSAACDALDQHNLKQNDQPMDILQIINCLTTIYDRLEQEHNNLVNVPLCVDMCLNWLLNVYDTGRTGRIRVLSFKTGIISLCKAHLEDKYRYLFKQVASSTGFCDQRRLGLLLHDSIQIPRQLGEVASFGGSNIEPSVRSCFQFANNKPEIEAALFLDWMRLEPQSMVWLPVLHRVAAAETAKHQAKCNICKECPIIGFRYRSLKHFNYDICQSCFFSGRVAKGHKMHYPMVEYCTPTTSGEDVRDFAKVLKNKFRTKRYFAKHPRMGYLPVQTVLEGDNMETPVTLINFWPVDSAPASSPQLSHDDTHSRIEHYASRLAEMENSNGSYLNDSISPNESIDDEHLLIQHYCQSLNQDSPLSQPRSPAQILISLESEERGELERILADLEEENRNLQAEYDRLKQQHEHKGLSPLPSPPEMMPTSPQSPRDAELIAEAKLLRQHKGRLEARMQILEDHNKQLESQLHRLRQLLEQPQAEAKVNGTTVSSPSTSLQRSDSSQPMLLRVVGSQTSDSMGEEDLLSPPQDTSTGLEEVMEQLNNSFPSSRGRNTPGKPMREDTM

SEQ ID NO: 26 - DNA, 3978 bp, Artificial Sequence
  Non-codon optimized Dys3978 gene
atgctttggtgggaagaagtagaggactgttatgaaagagaagatgttcaaaagaaaacattcacaaaatgggtaaatgcacaattttctaagtttgggaagcagcatattgagaacctcttcagtgacctacaggatgggaggcgcctcctagacctcctcgaaggcctgacagggcaaaaactgccaaaagaaaaaggatccacaagagttcatgccctgaacaatgtcaacaaggcactgcgggttttgcagaacaataatgttgatttagtgaatattggaagtactgacatcgtagatggaaatcataaactgactcttggtttgatttggaatataatcctccactggcaggtcaaaaatgtaatgaaaaatatcatggctggattgcaacaaaccaacagtgaaaagattctcctgagctgggtccgacaatcaactcgtaattatccacaggttaatgtaatcaacttcaccaccagctggtctgatggcctggctttgaatgctctcatccatagtcataggccagacctatttgactggaatagtgtggtttgccagcagtcagccacacaacgactggaacatgcattcaacatcgccagatatcaattaggcatagagaaactactcgatcctgaagatgttgataccacctatccagataagaagtccatcttaatgtacatcacatcactcttccaagttttgcctcaacaagtgagcattgaagccatccaggaagtggaaatgttgccaaggccacctaaagtgactaaagaagaacattttcagttacatcatcaaatgcactattctcaacagatcacggtcagtctagcacagggatatgagagaacttcttcccctaagcctcgattcaagagctatgcctacacacaggctgcttatgtcaccacctctgaccctacacggagcccatttccttcacagcatttggaagctcctgaagacaagtcatttggcagttcattgatggagagtgaagtaaacctggaccgttatcaaacagctttagaagaagtattatcgtggcttctttctgctgaggacacattgcaagcacaaggagagatttctaatgatgtggaagtggtgaaagaccagtttcatactcatgaggggtacatgatggatttgacagcccatcagggccgggttggtaatattctacaattgggaagtaagctgattggaacaggaaaattatcagaagatgaagaaactgaagtacaagagcagatgaatctcctaaattcaagatgggaatgcctcagggtagctagcatggaaaaacaaagcaatttacatagagttttaatggatctccagaatcagaaactgaaagagttgaatgactggctaacaaaaacagaagaaagaacaaggaaaatggaggaagagcctcttggacctgatcttgaagacctaaaacgccaagtacaacaacataaggtgcttcaagaagatctagaacaagaacaagtcagggtcaattctctcactcacatggtggtggtagttgatgaatctagtggagatcacgcaactgctgctttggaagaacaacttaaggtattgggagatcgatgggcaaacatctgtagatggacagaagaccgctgggttcttttacaagaccagcctgacctagctcctggactgaccactattggagcctctcctactcagactgttactctggtgacacaacctgtggttactaaggaaactgccatctccaaactagaaatgccatcttccttgatgttggaggtacctactcatagattactgcaacagttccccctggacctggaaaagtttcttgcctggcttacagaagctgaaacaactgccaatgtcctacaggatgctacccgtaaggaaaggctcctagaagactccaagggagtaaaagagctgatgaaacaatggcaagacctccaaggtgaaattgaagctcacacagatgtttatcacaacctggatgaaaacagccaaaaaatcctgagatccctggaaggttccgatgatgcagtcctgttacaaagacgtttggataacatgaacttcaagtggagtgaacttcggaaaaagtctctcaacattaggtcccatttggaagccagttctgaccagtggaagcgtctgcacctttctctgcaggaacttctggtgtggctacagctgaaagatgatgaattaagccggcaggcacctattggaggcgactttccagcagttcagaagcagaacgatgtacatagggccttcaagagggaattgaaaactaaagaacctgtaatcatgagtactcttgagactgtacgaatatttctgacagagcagcctttggaaggactagagaaactctaccaggagcccagagagctgcctcctgaggagagagcccagaatgtcactcggcttctacgaaagcaggctgaggaggtcaatactgagtgggaaaaattgaacctgcactccgctgactggcagagaaaaatagatgagacccttgaaagactccaggaacttcaagaggccacggatgagctggacctcaagctgcgccaagctgaggtgatcaagggatcctggcagcccgtgggcgatctcctcattgactctctccaagatcacctcgagaaagtcaaggcacttcgaggagaaattgcgcctctgaaagagaacgtgagccacgtcaatgaccttgctcgccagcttaccactttgggcattcagctctcaccgtataacctcagcactctggaagacctgaacaccagatggaagcttctgcaggtggccgtcgaggaccgagtcaggcagctgcatgaagcccacagggactttggtccagcatctcagcactttctttccacgtctgtccagggtccctgggagagagccatctcgccaaacaaagtgccctactatatcaaccacgagactcaaacaacttgctgggaccatcccaaaatgacagagctctaccagtctttagctgacctgaataatgtcagattctcagcttataggactgccatgaaactccgaagactgcagaaggccctttgcttggatctcttgagcctgtcagctgcatgtgatgccttggaccagcacaacctcaagcaaaatgaccagcccatggatatcctgcagattattaattgtttgaccactatttatgaccgcctggagcaagagcacaacaatttggtcaacgtccctctctgcgtggatatgtgtctgaactggctgctgaatgtttatgatacgggacgaacagggaggatccgtgtcctgtcttttaaaactggcatcatttccctgtgtaaagcacatttggaagacaagtacagataccttttcaagcaagtggcaagttcaacaggattttgtgaccagcgcaggctgggcctccttctgcatgattctatccaaattccaagacagttgggtgaagttgcatcctttgggggcagtaacattgagccaagtgtccggagctgcttccaatttgctaataataagccagagatcgaagcggccctcttcctagactggatgagactggaaccccagtccatggtgtggctgcccgtcctgcacagagtggctgctgcagaaactgccaagcatcaggccaaatgtaacatctgcaaagagtgtccaatcattggattcaggtacaggagtctaaagcactttaattatgacatctgccaaagctgctttttttctggtcgagttgcaaaaggccataaaatgcactatcccatggtggaatattgcactccgactacatcaggagaagatgttcgagactttgccaaggtactaaaaaacaaatttcgaaccaaaaggtattttgcgaagcatccccgaatgggctacctgccagtgcagactgtcttagagggggacaacatggaaacttag

SEQ ID NO: 27 - protein, 1329 aa, Artificial Sequence
  Delta3990 protein
MVWWEEVEDCYEREDVQKKTFTKWVNAQFSKFGKQHIENLFSDLQDGRRLLDLLEGLTGQKLPKEKGSTRVHALNNVNKALRVLQNNNVDLVNIGSTDIVDGNHKLTLGLIWNIILHWQVKNVMKNIMAGLQQTNSEKILLSWVRQSTRNYPQVNVINFTTSWSDGLALNALIHSHRPDLFDWNSVVCQQSATQRLEHAFNIARYQLGIEKLLDPEDVDTTYPDKKSILMYITSLFQVLPQQVSIEAIQEVEMLPRPPKVTKEEHFQLHHQMHYSQQITVSLAQGYERTSSPKPRFKSYAYTQAAYVTTSDPTRSPFPSQHLEAPEDKSFGSSLMESEVNLDRYQTALEEVLSWLLSAEDTLQAQGEISNDVEVVKDQFHTHEGYMMDLTAHQGRVGNILQLGSKLIGTGKLSEDEETEVQEQMNLLNSRWECLRVASMEKQSNLHRVLMDLQNQKLKELNDWLTKTEERTRKMEEEPLGPDLEDLKRQVQQHKVLQEDLEQEQVRVNSLTHMVVVVDESSGDHATAALEEQLKVLGDRWANICRWTEDRWVLLQDQPDLAPGLTTIGASPTQTVTLVTQPVVTKETAISKLEMPSSLMLEVPTHRLLQQFPLDLEKFLAWLTEAETTANVLQDATRKERLLEDSKGVKELMKQWQDLQGEIEAHTDVYHNLDENSQKILRSLEGSDDAVLLQRRLDNMNFKWSELRKKSLNIRSHLEASSDQWKRLHLSLQELLVWLQLKDDELSRQAPIGGDFPAVQKQNDVHRAFKRELKTKEPVIMSTLETVRIFLTEQPLEGLEKLYQEPRELPPEERAQNVTRLLRKQAEEVNTEWEKLNLHSADWQRKIDETLERLQELQEATDELDLKLRQAEVIKGSWQPVGDLLIDSLQDHLEKVKALRGEIAPLKENVSHVNDLARQLTTLGIQLSPYNLSTLEDLNTRWKLLQVAVEDRVRQLHEAHRDFGPASQHFLSTSVQGPWERAISPNKVPYYINHETQTTCWDHPKMTELYQSLADLNNVRFSAYRTAMKLRRLQKALCLDLLSLSAACDALDQHNLKQNDQPMDILQIINCLTTIYDRLEQEHNNLVNVPLCVDMCLNWLLNVYDTGRTGRIRVLSFKTGIISLCKAHLEDKYRYLFKQVASSTGFCDQRRLGLLLHDSIQIPRQLGEVASFGGSNIEPSVRSCFQFANNKPEIEAALFLDWMRLEPQSMVWLPVLHRVAAAETAKHQAKCNICKECPIIGFRYRSLKHFNYDICQSCFFSGRVAKGHKMHYPMVEYCTPTTSGEDVRDFAKVLKNKFRTKRYFAKHPRMGYLPVQTVLEGDNMETPDTM

SEQ ID NO: 28 - DNA, 3990 bp, Artificial Sequence
  Delta3990 gene
atggtttggtgggaagaagtagaggactgttatgaaagagaagatgttcaaaagaaaacattcacaaaatgggtaaatgcacaattttctaagtttgggaagcagcatattgagaacctcttcagtgacctacaggatgggaggcgcctcctagacctcctcgaaggcctgacagggcaaaaactgccaaaagaaaaaggatccacaagagttcatgccctgaacaatgtcaacaaggcactgcgggttttgcagaacaataatgttgatttagtgaatattggaagtactgacatcgtagatggaaatcataaactgactcttggtttgatttggaatataatcctccactggcaggtcaaaaatgtaatgaaaaatatcatggctggattgcaacaaaccaacagtgaaaagattctcctgagctgggtccgacaatcaactcgtaattatccacaggttaatgtaatcaacttcaccaccagctggtctgatggcctggctttgaatgctctcatccatagtcataggccagacctatttgactggaatagtgtggtttgccagcagtcagccacacaacgactggaacatgcattcaacatcgccagatatcaattaggcatagagaaactactcgatcctgaagatgttgataccacctatccagataagaagtccatcttaatgtacatcacatcactcttccaagttttgcctcaacaagtgagcattgaagccatccaggaagtggaaatgttgccaaggccacctaaagtgactaaagaagaacattttcagttacatcatcaaatgcactattctcaacagatcacggtcagtctagcacagggatatgagagaacttcttcccctaagcctcgattcaagagctatgcctacacacaggctgcttatgtcaccacctctgaccctacacggagcccatttccttcacagcatttggaagctcctgaagacaagtcatttggcagttcattgatggagagtgaagtaaacctggaccgttatcaaacagctttagaagaagtattatcgtggcttctttctgctgaggacacattgcaagcacaaggagagatttctaatgatgtggaagtggtgaaagaccagtttcatactcatgaggggtacatgatggatttgacagcccatcagggccgggttggtaatattctacaattgggaagtaagctgattggaacaggaaaattatcagaagatgaagaaactgaagtacaagagcagatgaatctcctaaattcaagatgggaatgcctcagggtagctagcatggaaaaacaaagcaatttacatagagttttaatggatctccagaatcagaaactgaaagagttgaatgactggctaacaaaaacagaagaaagaacaaggaaaatggaggaagagcctcttggacctgatcttgaagacctaaaacgccaagtacaacaacataaggtgcttcaagaagatctagaacaagaacaagtcagggtcaattctctcactcacatggtggtggtagttgatgaatctagtggagatcacgcaactgctgctttggaagaacaacttaaggtattgggagatcgatgggcaaacatctgtagatggacagaagaccgctgggttcttttacaagaccagcctgacctagctcctggactgaccactattggagcctctcctactcagactgttactctggtgacacaacctgtggttactaaggaaactgccatctccaaactagaaatgccatcttccttgatgttggaggtacctactcatagattactgcaacagttccccctggacctggaaaagtttcttgcctggcttacagaagctgaaacaactgccaatgtcctacaggatgctacccgtaaggaaaggctcctagaagactccaagggagtaaaagagctgatgaaacaatggcaagacctccaaggtgaaattgaagctcacacagatgtttatcacaacctggatgaaaacagccaaaaaatcctgagatccctggaaggttccgatgatgcagtcctgttacaaagacgtttggataacatgaacttcaagtggagtgaacttcggaaaaagtctctcaacattaggtcccatttggaagccagttctgaccagtggaagcgtctgcacctttctctgcaggaacttctggtgtggctacagctgaaagatgatgaattaagccggcaggcacctattggaggcgactttccagcagttcagaagcagaacgatgtacatagggccttcaagagggaattgaaaactaaagaacctgtaatcatgagtactcttgagactgtacgaatatttctgacagagcagcctttggaaggactagagaaactctaccaggagcccagagagctgcctcctgaggagagagcccagaatgtcactcggcttctacgaaagcaggctgaggaggtcaatactgagtgggaaaaattgaacctgcactccgctgactggcagagaaaaatagatgagacccttgaaagactccaggaacttcaagaggccacggatgagctggacctcaagctgcgccaagctgaggtgatcaagggatcctggcagcccgtgggcgatctcctcattgactctctccaagatcacctcgagaaagtcaaggcacttcgaggagaaattgcgcctctgaaagagaacgtgagccacgtcaatgaccttgctcgccagcttaccactttgggcattcagctctcaccgtataacctcagcactctggaagacctgaacaccagatggaagcttctgcaggtggccgtcgaggaccgagtcaggcagctgcatgaagcccacagggactttggtccagcatctcagcactttctttccacgtctgtccagggtccctgggagagagccatctcgccaaacaaagtgccctactatatcaaccacgagactcaaacaacttgctgggaccatcccaaaatgacagagctctaccagtctttagctgacctgaataatgtcagattctcagcttataggactgccatgaaactccgaagactgcagaaggccctttgcttggatctcttgagcctgtcagctgcatgtgatgccttggaccagcacaacctcaagcaaaatgaccagcccatggatatcctgcagattattaattgtttgaccactatttatgaccgcctggagcaagagcacaacaatttggtcaacgtccctctctgcgtggatatgtgtctgaactggctgctgaatgtttatgatacgggacgaacagggaggatccgtgtcctgtcttttaaaactggcatcatttccctgtgtaaagcacatttggaagacaagtacagataccttttcaagcaagtggcaagttcaacaggattttgtgaccagcgcaggctgggcctccttctgcatgattctatccaaattccaagacagttgggtgaagttgcatcctttgggggcagtaacattgagccaagtgtccggagctgcttccaatttgctaataataagccagagatcgaagcggccctcttcctagactggatgagactggaaccccagtccatggtgtggctgcccgtcctgcacagagtggctgctgcagaaactgccaagcatcaggccaaatgtaacatctgcaaagagtgtccaatcattggattcaggtacaggagtctaaagcactttaattatgacatctgccaaagctgctttttttctggtcgagttgcaaaaggccataaaatgcactatcccatggtggaatattgcactccgactacatcaggagaagatgttcgagactttgccaaggtactaaaaaacaaatttcgaaccaaaaggtattttgcgaagcatccccgaatgggctacctgccagtgcagactgtcttagagggggacaacatggaaactcccgacacaatgtag